European Patent Application EP 4 534 556 A1, published April 9, 2025. Title: CHIMERIC ANTIGEN RECEPTOR CONTAINING CLDN18.2 SINGLE DOMAIN ANTIBODY AND APPLICATION THEREOF. Applicant: SUZHOU IMMUNOFOCO BIOTECHNOLOGY CO. LTD. The sequence listing filed with the application follows.

SEQUENCE LISTING (19 sequences)

SEQ ID NO: 1 - protein, 5 aa, synthetic construct
  REGION 1..5: note = CDR1 of CLDN18.2 VHH
IPVMG

SEQ ID NO: 2 - protein, 16 aa, synthetic construct
  REGION 1..16: note = CDR3 of CLDN18.2 VHH
GISTGGTTNYGDSVKG

SEQ ID NO: 3 - protein, 12 aa, synthetic construct
  REGION 1..12: note = CDR3 of CLDN18.2 VHH
LVVSGIGSTLEV

SEQ ID NO: 4 - protein, 120 aa, synthetic construct
  REGION 1..120: note = humanized CLDN18.2 VHH full length
QVQLVESGGGLVQPGGSLRLSCAASGSIFNIPVMGWYRQAPGKQRELVAGISTGGTTNYGDSVKGRFTISRDNAKNTVYLQMNSLKPEDTAVYYCNVLVVSGIGSTLEVWGQGTLVTVSS

SEQ ID NO: 5 - protein, 361 aa, synthetic construct
  REGION 1..361: note = CAR full length
MLLLVTSLLLCELPHPAFLLIPQVQLVESGGGLVQPGGSLRLSCAASGSIFNIPVMGWYRQAPGKQRELVAGISTGGTTNYGDSVKGRFTISRDNAKNTVYLQMNSLKPEDTAVYYCNVLVVSGIGSTLEVWGQGTLVTVSSIEVMYPPPYLDNEKSNGTIIHVKGKHLCPSPLFPGPSKPFWVLVVVGGVLACYSLLVTVAFIIFWVRSKRSRLLHSDYMNMTPRRPGPTRKHYQPYAPPRDFAAYRSRVKFSRSADAPAYQQGQNQLYNELNLGRREEYDVLDKRRGRDPEMGGKPRRKNPQEGLYNELQKDKMAEAYSEIGMKGERRRGKGHDGLYQGLSTATKDTYDALHMQALPPR

SEQ ID NO: 6 - protein, 39 aa, synthetic construct
  REGION 1..39: note = CD28 hinge
IEVMYPPPYLDNEKSNGTIIHVKGKHLCPSPLFPGPSKP

SEQ ID NO: 7 - protein, 15 aa, synthetic construct
  REGION 1..15: note = short CD28 hinge
KHLCPSPLFPGPSKP

SEQ ID NO: 8 - protein, 45 aa, synthetic construct
  REGION 1..45: note = CD8 hinge
TTTPAPRPPTPAPTIASQPLSLRPEACRPAAGGAVHTRGLDFACD

SEQ ID NO: 9 - protein, 27 aa, synthetic construct
  REGION 1..27: note = transmembrane region of CD28
FWVLVVVGGVLACYSLLVTVAFIIFWV

SEQ ID NO: 10 - protein, 24 aa, synthetic construct
  REGION 1..24: note = transmembrane region of CD8
IYIWAPLAGTCGVLLLSLVITLYC

SEQ ID NO: 11 - protein, 112 aa, synthetic construct
  REGION 1..112: note = CD3 signal transduction domain
RVKFSRSADAPAYQQGQNQLYNELNLGRREEYDVLDKRRGRDPEMGGKPRRKNPQEGLYNELQKDKMAEAYSEIGMKGERRRGKGHDGLYQGLSTATKDTYDALHMQALPPR

SEQ ID NO: 12 - protein, 41 aa, synthetic construct
  REGION 1..41: note = CD28 signal transduction domain
RSKRSRLLHSDYMNMTPRRPGPTRKHYQPYAPPRDFAAYRS

SEQ ID NO: 13 - protein, 42 aa, synthetic construct
  REGION 1..42: note = OX40 signal transduction domain
ALYLLRRDQRLPPDAHKPPGGGSFRTPIQEEQADAHSTLAKI

SEQ ID NO: 14 - protein, 42 aa, synthetic construct
  REGION 1..42: note = 4-1BB signal transduction domain
KRGRKKLLYIFKQPFMRPVQTTQEEDGCSCRFPEEEEGGCEL

SEQ ID NO: 15 - protein, 38 aa, synthetic construct
  REGION 1..38: note = ICOS signal transduction domain
CWLTKKKYSSSVHDPNGEYMFMRAVNTAKKSRLTDVTL

SEQ ID NO: 16 - protein, 121 aa, synthetic construct
  REGION 1..121: note = humanized CLDN18.2 VHH full length
EVQLVESGGGLVQPGGSLRLSCAASGNIFRGDIMTWYRQAPGKGRELVAATTGDSITGRGSYKGVRFTISRDNAKNTLYLQMNSLRAEDTAVYYCNAGPWDYLTARQVFEWGQGTLVTVSS

SEQ ID NO: 17 - protein, 121 aa, synthetic construct
  REGION 1..121: note = humanized CLDN18.2 VHH full length
EVQVVESGGGLVQPGGSLRLSCAASGNIFRTDIGMWYRQAPGKGRELVAGTTTGRSGYVDKASIGRFTISRDNAKNTMYLQMNSLRAEDTAVYYCNAYGVWEQTPFDALRWGQGTLVTVSS

SEQ ID NO: 18 - protein, 123 aa, synthetic construct
  REGION 1..123: note = humanized CLDN18.2 VHH full length
EVQLVESGGGLVQPGGSLRLSCAASGSIFSVNGIMWYRQAPGKQRELVAARYTGSVIDSGKTGTGRFTISRDNAKNTLYLQMNSLRAEDTAVYYCNAPTAALTRVEWDVYSLWGQGTLVTVSS

SEQ ID NO: 19 - protein, 246 aa, synthetic construct
  REGION 1..246: note = CLDN18.2 scfv full length
QVQLQQPGAELVRPGASVKLSCKASGYTFTSYWINWVKQRPGQGLEWIGNIYPSDSYTNYNQKFKDKATLTVDKSSSTAYMQLSSPTSEDSAVYYCTRSWRGNSFDYWGQGTTLTVSSGGGGSGGGGSGGGGSDIVMTQSPSSLTVTAGEKVTMSCKSSQSLLNSGNQKNYLTWYQQKPGQPPKLLIYWASTRESGVPDRFTGSGSGTDFTLTISSVQAEDLAVYYCQNDYSYPFTFGSGTKLEIK